European Patent Application EP 4 644 566 A1, published November 5, 2025. Title: IMPROVED NUCLEIC ACID CAPTURE METHOD. Applicant: BGI SHENZHEN. The sequence listing filed with the application follows.

SEQUENCE LISTING (3 sequences)

SEQ ID NO: 1 - DNA, 22 bp, synthetic construct
  source 1..22: mol_type = other DNA
ttgtcttcctaagaccgcttgg

SEQ ID NO: 2 - DNA, 44 bp, synthetic construct
  source 1..44: mol_type = other DNA
cctccgactgtgtgacttagacttgcacttgatgtgctnnnnnn

SEQ ID NO: 3 - DNA, 45 bp, synthetic construct
  source 1..45: mol_type = other DNA
caagtgcaagtctaagtcacacagtcggaggccaagcggtcttag